European Patent Application EP 4 491 707 A1, published January 15, 2025. Title: Microorganism comprising Geranylgeranyl pyrophosphate synthase derived from Dunaliella salina, for producing carotenoid or compound in which a precursor thereof is carotenoid, and method using the same. Applicant: 씨제이제일제당 주식회사. Application KR. The sequence listing filed with the application follows.

SEQUENCE LISTING (91 sequences)

SEQ ID NO: 1 - DNA, 1074 bp, synthetic construct
  source 1..1074: mol_type = other DNA
atggctgcccaccagatgcagctcctaaactcccagcgattgtgctctacctcgacgcgtagtattagacctgctgtcagcaaccgaccccaggtgccacgcaggcctgccaacgtgagacgggggcgttaccaggcctgccgaaccatggccatcgccactgcagatgaggccaagcagtctacttcgtccttcgatttccagggctacatgatggagcgggccgtgatggtcaatgatgccctcgacaaggctcttccgcaaagacaccctgaggttttactggacgccatgcgttattcacttctcgctggaggcaaaagagttcggccggctctcacactcgccgcttgtgagttggtgggcggcgatattgcatgtgccatgcccaccgcatgcgctatggaagtcgtgcataccatgtctttgatccacgatgatctgccctccatggataatgacgactttcggcgaggtcgaccaacaaaccacaaggtctacggagaggatattgcgatattagccggcgacgcgctattgtcgtttgcctttgagcacgtagcacgcgctaccaccggtactagccctgaacgagtactccgagtgattcttgagctcggcaaggccgttggtgcagacgggctgactggtggacaggtggtggacatcaagtctgagaacgaggaagtgggcctggaggttctgcaatacatccatgagcataaaacagcggccctgctcgaagcctcagtcgtttgtggagcactggtcggtggagcggacgatgtgactgttgagaaactgcgaaagtacgctcgaaacattggcctggccttccaagttgtcgacgacatccttgactgcacccagacgaccgagatgctgggaaagacggcgggaaaggacattgacgtcaacaaaaccacgtaccccaagctgctgggtctcgaaaagtccaagcaggcagctgaagacctcattgctgaggctatccagcagctggacggcttcccccccgagaagcgaactcctcttgtggctcttgctaagtatatcggataccgacagaactga

SEQ ID NO: 2 - DNA, 531 bp, synthetic construct
  source 1..531: mol_type = other DNA
agagaccgggttggcggcgcatttgtgtcccaaaaaacagccccaattgccccaattgaccccaaattgacccagtagcgggcccaaccccggcgagagcccccttctccccacatatcaaacctcccccggttcccacacttgccgttaagggcgtagggtactgcagtctggaatctacgcttgttcagactttgtactagtttctttgtctggccatccgggtaacccatgccggacgcaaaatagactactgaaaatttttttgctttgtggttgggactttagccaagggtataaaagaccaccgtccccgaattacctttcctcttcttttctctctctccttgtcaactcacacccgaaatcgttaagcatttccttctgagtataagaatcattcaaaatggtgagtttcagaggcagcagcaattgccacgggctttgagcacacggccgggtgtggtcccattcccatcgacacaagacgccacgtcatccgaccagcactttttgcagtactaaccgcag

SEQ ID NO: 3 - DNA, 500 bp, synthetic construct
  source 1..500: mol_type = other DNA
ctatccgaagatcaagagcgaagcaagttgtaagtccaggacatgtttcccgcccacgcgagtgatttataacacctctcttttttgacacccgctcgccttgaaattcatgtcacataaattatagtcaacgacgtttgaataacttgtcttgtagttcgatgatgatcatatgattacattaatagtaattactgtatttgatatatatactaattacaatagtacatattagaacatacaatagttagtgccgtgaagtggcttaaaataccgcgagtcgattacgtaatattatatataatgtcaaagtggggtcccagagccgaagaaggtgcttttcttgaagatcccagtgtattggacaagtatatctgtctctatgattgtttttccaggtgaaaatgttgaacaaagtgtctactggagtttgtaagcgctggtgcgactggggccacttttaaaacccgccttagcaggctttttcaccgttccaagac

SEQ ID NO: 4 - DNA, 2102 bp, synthetic construct
  source 1..2102: mol_type = other DNA
agagaccgggttggcggcgcatttgtgtcccaaaaaacagccccaattgccccaattgaccccaaattgacccagtagcgggcccaaccccggcgagagcccccttctccccacatatcaaacctcccccggttcccacacttgccgttaagggcgtagggtactgcagtctggaatctacgcttgttcagactttgtactagtttctttgtctggccatccgggtaacccatgccggacgcaaaatagactactgaaaatttttttgctttgtggttgggactttagccaagggtataaaagaccaccgtccccgaattacctttcctcttcttttctctctctccttgtcaactcacacccgaaatcgttaagcatttccttctgagtataagaatcattcaaaatggtgagtttcagaggcagcagcaattgccacgggctttgagcacacggccgggtgtggtcccattcccatcgacacaagacgccacgtcatccgaccagcactttttgcagtactaaccgcaggctgcccaccagatgcagctcctaaactcccagcgattgtgctctacctcgacgcgtagtattagacctgctgtcagcaaccgaccccaggtgccacgcaggcctgccaacgtgagacgggggcgttaccaggcctgccgaaccatggccatcgccactgcagatgaggccaagcagtctacttcgtccttcgatttccagggctacatgatggagcgggccgtgatggtcaatgatgccctcgacaaggctcttccgcaaagacaccctgaggttttactggacgccatgcgttattcacttctcgctggaggcaaaagagttcggccggctctcacactcgccgcttgtgagttggtgggcggcgatattgcatgtgccatgcccaccgcatgcgctatggaagtcgtgcataccatgtctttgatccacgatgatctgccctccatggataatgacgactttcggcgaggtcgaccaacaaaccacaaggtctacggagaggatattgcgatattagccggcgacgcgctattgtcgtttgcctttgagcacgtagcacgcgctaccaccggtactagccctgaacgagtactccgagtgattcttgagctcggcaaggccgttggtgcagacgggctgactggtggacaggtggtggacatcaagtctgagaacgaggaagtgggcctggaggttctgcaatacatccatgagcataaaacagcggccctgctcgaagcctcagtcgtttgtggagcactggtcggtggagcggacgatgtgactgttgagaaactgcgaaagtacgctcgaaacattggcctggccttccaagttgtcgacgacatccttgactgcacccagacgaccgagatgctgggaaagacggcgggaaaggacattgacgtcaacaaaaccacgtaccccaagctgctgggtctcgaaaagtccaagcaggcagctgaagacctcattgctgaggctatccagcagctggacggcttcccccccgagaagcgaactcctcttgtggctcttgctaagtatatcggataccgacagaactgactatccgaagatcaagagcgaagcaagttgtaagtccaggacatgtttcccgcccacgcgagtgatttataacacctctcttttttgacacccgctcgccttgaaattcatgtcacataaattatagtcaacgacgtttgaataacttgtcttgtagttcgatgatgatcatatgattacattaatagtaattactgtatttgatatatatactaattacaatagtacatattagaacatacaatagttagtgccgtgaagtggcttaaaataccgcgagtcgattacgtaatattatatataatgtcaaagtggggtcccagagccgaagaaggtgcttttcttgaagatcccagtgtattggacaagtatatctgtctctatgattgtttttccaggtgaaaatgttgaacaaagtgtctactggagtttgtaagcgctggtgcgactggggccacttttaaaacccgccttagcaggctttttcaccgttccaagac

SEQ ID NO: 5 - DNA, 1533 bp, Yarrowia lipolytica
  source 1..1533: mol_type = genomic DNA
tgcctcctgtctgactcgtcattgccgcctttggagtacgactccaactatgagtgtgcttggatcactttgacgatacattcttcgttggaggctgtgggtctgacagctgcgttttcggcgcggttggccgacaacaatatcagctgcaacgtcattgctggctttcatcatgatcacatttttgtcggcaaaggcgacgcccagagagccattgacgttctttctaatttggaccgatagccgtatagtccagtctatctataagttcaactaactcgtaactattaccataacatatacttcactgccccagataaggttccgataaaaagttctgcagactaaatttatttcagtctcctcttcaccaccaaaatgccctcctacgaagctcgagctaacgtccacaagtccgcctttgccgctcgagtgctcaagctcgtggcagccaagaaaaccaacctgtgtgcttctctggatgttaccaccaccaaggagctcattgagcttgccgataaggtcggaccttatgtgtgcatgatcaagacccatatcgacatcattgacgacttcacctacgccggcactgtgctccccctcaaggaacttgctcttaagcacggtttcttcctgttcgaggacagaaagttcgcagatattggcaacactgtcaagcaccagtacaagaacggtgtctaccgaatcgccgagtggtccgatatcaccaacgcccacggtgtacccggaaccggaatcattgctggcctgcgagctggtgccgaggaaactgtctctgaacagaagaaggaggacgtctctgactacgagaactcccagtacaaggagttcctggtcccctctcccaacgagaagctggccagaggtctgctcatgctggccgagctgtcttgcaagggctctctggccactggcgagtactccaagcagaccattgagcttgcccgatccgaccccgagtttgtggttggcttcattgcccagaaccgacctaagggcgactctgaggactggcttattctgacccccggggtgggtcttgacgacaagggagacgctctcggacagcagtaccgaactgttgaggatgtcatgtctaccggaacggatatcataattgtcggccgaggtctgtacggccagaaccgagatcctattgaggaggccaagcgataccagaaggctggctgggaggcttaccagaagattaactgttagaggttagactatggatatgtcatttaactgtgtatatagagagcgtgcaagtatggagcgcttgttcagcttgtatgatggtcagacgacctgtctgatcgagtatgtatgatactgcacaacctgtgtatccgcatgatctgtccaatggggcatgttgttgtgtttctcgatacggagatgctgggtacaagtagctaatacgattgaactacttatacttatatgaggcttgaagaaagctgacttgtgtatgacttattctcaactacatccccagtcacaataccacca

SEQ ID NO: 6 - DNA, 1131 bp, synthetic construct
  source 1..1131: mol_type = other DNA
atggattacgcgaacatcctcacagcaattccactcgagtttactcctcaggatgatatcgtgctccttgaaccgtatcactacctaggaaagaaccctggaaaagaaattcgatcacaactcatcgaggctttcaactattggttggatgtcaagaaggaggatctcgaggtcatccagaacgttgttggcatgctacataccgctagcttattaatggacgatgtggaggattcatcggtcctcaggcgtgggtcgcctgtagcccatctaatttacgggattccgcagacaataaacactgcaaactacgtctactttctggcttatcaagagatcttcaagcttcgcccaacaccgatacccatgcctgtaattcctccttcatctgcttcgcttcaatcaaccgtctcctctgcatcctcctcctcctcggcctcgtctgaaaacgggggcacgtcatctcctaattcgcagattccgttctcgaaagatacgtatcttgataaagtgatcacagacgagatgctttccctccatagagggcaaggcctggagctattctggagagatagtctgacgtgtcctagcgaagaggaatatgtgaaaatggttcttggaaagacgggaggtttgttccgtatagcggtcagattgatgatggcaaagtcagaatgtgacatagactttgtccagcttgtcaacttgatctcaatatacttccagatcagggatgactatatgaaccttcagtcttctgagtatgcccatattaagaattttgcagaggacctcacagaaggaaaattcagttttcccactatccactcgattcgtgccaacccctcatcgagactcgtcatcaatacgttgcagaagaaatcgacctctcctgagatccttcaccactgtgtaaactacatgcgcacagaaacccactcattcgaatatactcaggaagtcctcaacaccttgtcaggtgcactcgagagagaactaggaaggcttcaaggagagttcgcagaagctaactcaaagattgatcttggagacgtagagtcggaaggaagaacggggaagaacgtcaaattggaagcgatcctgaaaaagctagccgatatccctctgtga

SEQ ID NO: 7 - DNA, 2159 bp, synthetic construct
  source 1..2159: mol_type = other DNA
agagaccgggttggcggcgcatttgtgtcccaaaaaacagccccaattgccccaattgaccccaaattgacccagtagcgggcccaaccccggcgagagcccccttctccccacatatcaaacctcccccggttcccacacttgccgttaagggcgtagggtactgcagtctggaatctacgcttgttcagactttgtactagtttctttgtctggccatccgggtaacccatgccggacgcaaaatagactactgaaaatttttttgctttgtggttgggactttagccaagggtataaaagaccaccgtccccgaattacctttcctcttcttttctctctctccttgtcaactcacacccgaaatcgttaagcatttccttctgagtataagaatcattcaaaatggtgagtttcagaggcagcagcaattgccacgggctttgagcacacggccgggtgtggtcccattcccatcgacacaagacgccacgtcatccgaccagcactttttgcagtactaaccgcaggattacgcgaacatcctcacagcaattccactcgagtttactcctcaggatgatatcgtgctccttgaaccgtatcactacctaggaaagaaccctggaaaagaaattcgatcacaactcatcgaggctttcaactattggttggatgtcaagaaggaggatctcgaggtcatccagaacgttgttggcatgctacataccgctagcttattaatggacgatgtggaggattcatcggtcctcaggcgtgggtcgcctgtagcccatctaatttacgggattccgcagacaataaacactgcaaactacgtctactttctggcttatcaagagatcttcaagcttcgcccaacaccgatacccatgcctgtaattcctccttcatctgcttcgcttcaatcaaccgtctcctctgcatcctcctcctcctcggcctcgtctgaaaacgggggcacgtcatctcctaattcgcagattccgttctcgaaagatacgtatcttgataaagtgatcacagacgagatgctttccctccatagagggcaaggcctggagctattctggagagatagtctgacgtgtcctagcgaagaggaatatgtgaaaatggttcttggaaagacgggaggtttgttccgtatagcggtcagattgatgatggcaaagtcagaatgtgacatagactttgtccagcttgtcaacttgatctcaatatacttccagatcagggatgactatatgaaccttcagtcttctgagtatgcccatattaagaattttgcagaggacctcacagaaggaaaattcagttttcccactatccactcgattcgtgccaacccctcatcgagactcgtcatcaatacgttgcagaagaaatcgacctctcctgagatccttcaccactgtgtaaactacatgcgcacagaaacccactcattcgaatatactcaggaagtcctcaacaccttgtcaggtgcactcgagagagaactaggaaggcttcaaggagagttcgcagaagctaactcaaagattgatcttggagacgtagagtcggaaggaagaacggggaagaacgtcaaattggaagcgatcctgaaaaagctagccgatatccctctgtgactatccgaagatcaagagcgaagcaagttgtaagtccaggacatgtttcccgcccacgcgagtgatttataacacctctcttttttgacacccgctcgccttgaaattcatgtcacataaattatagtcaacgacgtttgaataacttgtcttgtagttcgatgatgatcatatgattacattaatagtaattactgtatttgatatatatactaattacaatagtacatattagaacatacaatagttagtgccgtgaagtggcttaaaataccgcgagtcgattacgtaatattatatataatgtcaaagtggggtcccagagccgaagaaggtgcttttcttgaagatcccagtgtattggacaagtatatctgtctctatgattgtttttccaggtgaaaatgttgaacaaagtgtctactggagtttgtaagcgctggtgcgactggggccacttttaaaacccgccttagcaggctttttcaccgttccaagac

SEQ ID NO: 8 - DNA, 1008 bp, Saccharomyces cerevisiae
  source 1..1008: mol_type = genomic DNA
atggaggccaagatagatgagctgatcaataatgatcctgtttggtccagccaaaatgaaagcttgatttcaaaaccttataatcacatccttttgaaacctggcaagaactttagactaaatttaatagttcaaattaacagagttatgaatttgcccaaagaccagctggccatagtttcgcaaattgttgagctcttgcataattccagccttttaatcgacgatatagaagataatgctcccttgagaaggggacagaccacttctcacttaatcttcggtgtaccctccactataaacaccgcaaattatatgtatttcagagccatgcaacttgtatcgcagctaaccacaaaagagcctttgtatcataatttgattacgattttcaacgaagaattgatcaatctacataggggacaaggcttggatatatactggagagactttctgcctgaaatcatacctactcaggagatgtatttgaatatggttatgaataaaacaggcggccttttcagattaacgttgagactcatggaagcgctgtctccttcctcacaccacggccattcgttggttcctttcataaatcttctgggtattatttatcagattagagatgattacttgaatttgaaagatttccaaatgtccagcgaaaaaggctttgctgaggacattacagaggggaagttatcttttcccatcgtccacgcccttaacttcactaaaacgaaaggtcaaactgagcaacacaatgaaattctaagaattctcctgttgaggacaagtgataaagatataaaactaaagctgattcaaatactggaattcgacaccaattcattggcctacaccaaaaattttattaatcaattagtgaatatgataaaaaatgataatgaaaataagtatttacctgatttggcttcgcattccgacaccgccaccaatttacatgacgaattgttatatataatagaccacttatccgaattgtga

SEQ ID NO: 9 - DNA, 2036 bp, synthetic construct
  source 1..2036: mol_type = other DNA
agagaccgggttggcggcgcatttgtgtcccaaaaaacagccccaattgccccaattgaccccaaattgacccagtagcgggcccaaccccggcgagagcccccttctccccacatatcaaacctcccccggttcccacacttgccgttaagggcgtagggtactgcagtctggaatctacgcttgttcagactttgtactagtttctttgtctggccatccgggtaacccatgccggacgcaaaatagactactgaaaatttttttgctttgtggttgggactttagccaagggtataaaagaccaccgtccccgaattacctttcctcttcttttctctctctccttgtcaactcacacccgaaatcgttaagcatttccttctgagtataagaatcattcaaaatggtgagtttcagaggcagcagcaattgccacgggctttgagcacacggccgggtgtggtcccattcccatcgacacaagacgccacgtcatccgaccagcactttttgcagtactaaccgcaggaggccaagatagatgagctgatcaataatgatcctgtttggtccagccaaaatgaaagcttgatttcaaaaccttataatcacatccttttgaaacctggcaagaactttagactaaatttaatagttcaaattaacagagttatgaatttgcccaaagaccagctggccatagtttcgcaaattgttgagctcttgcataattccagccttttaatcgacgatatagaagataatgctcccttgagaaggggacagaccacttctcacttaatcttcggtgtaccctccactataaacaccgcaaattatatgtatttcagagccatgcaacttgtatcgcagctaaccacaaaagagcctttgtatcataatttgattacgattttcaacgaagaattgatcaatctacataggggacaaggcttggatatatactggagagactttctgcctgaaatcatacctactcaggagatgtatttgaatatggttatgaataaaacaggcggccttttcagattaacgttgagactcatggaagcgctgtctccttcctcacaccacggccattcgttggttcctttcataaatcttctgggtattatttatcagattagagatgattacttgaatttgaaagatttccaaatgtccagcgaaaaaggctttgctgaggacattacagaggggaagttatcttttcccatcgtccacgcccttaacttcactaaaacgaaaggtcaaactgagcaacacaatgaaattctaagaattctcctgttgaggacaagtgataaagatataaaactaaagctgattcaaatactggaattcgacaccaattcattggcctacaccaaaaattttattaatcaattagtgaatatgataaaaaatgataatgaaaataagtatttacctgatttggcttcgcattccgacaccgccaccaatttacatgacgaattgttatatataatagaccacttatccgaattgtgactatccgaagatcaagagcgaagcaagttgtaagtccaggacatgtttcccgcccacgcgagtgatttataacacctctcttttttgacacccgctcgccttgaaattcatgtcacataaattatagtcaacgacgtttgaataacttgtcttgtagttcgatgatgatcatatgattacattaatagtaattactgtatttgatatatatactaattacaatagtacatattagaacatacaatagttagtgccgtgaagtggcttaaaataccgcgagtcgattacgtaatattatatataatgtcaaagtggggtcccagagccgaagaaggtgcttttcttgaagatcccagtgtattggacaagtatatctgtctctatgattgtttttccaggtgaaaatgttgaacaaagtgtctactggagtttgtaagcgctggtgcgactggggccacttttaaaacccgccttagcaggctttttcaccgttccaagac

SEQ ID NO: 10 - DNA, 984 bp, Yarrowia lipolytica
  source 1..984: mol_type = genomic DNA
atggattataacagcgcggatttcaaggagatatggggcaaggccgccgacaccgcgctgctgggaccgtacaactacctcgccaacaaccggggccacaacatcagagaacacttgatcgcagcgttcggagcggttatcaaggtggacaagagcgatctcgagaccatttcgcacatcaccaagattttgcataactcgtcgctgcttgttgatgacgtggaagacaactcgatgctccgacgaggcctgccggcagcccattgtctgtttggagtcccccaaaccatcaactccgccaactacatgtactttgtggctctgcaggaggtgctcaagctcaagtcttatgatgccgtctccattttcaccgaggaaatgatcaacttgcatagaggtcagggtatggatctctactggagagaaacactcacttgcccctcggaagacgagtatctggagatggtggtgcacaagaccggtggactgtttcggctggctctgagacttatgctgtcggtggcatcgaaacaggaggaccatgaaaagatcaactttgatctcacacaccttaccgacacactgggagtcatttaccagattctggatgattacctcaacctgcagtccacggaattgaccgagaacaagggattctgcgaagatatcagcgaaggaaagttttcgtttccgctgattcacagcatacgcaccaacccggataaccacgagattctcaacattctcaaacagcgaacaagcgacgcttcactcaaaaagtacgccgtggactacatgagaacagaaaccaagagtttcgactactgcctcaagaggatacaggccatgtcactcaaggcaagttcgtacattgatgatctagcagcagctggccacgatgtctccaagctacgagccattttgcattattttgtgtccacctctgactgtgaggagagaaagtactttgaggatgcgcagtga

SEQ ID NO: 11 - DNA, 2012 bp, synthetic construct
  source 1..2012: mol_type = other DNA
agagaccgggttggcggcgcatttgtgtcccaaaaaacagccccaattgccccaattgaccccaaattgacccagtagcgggcccaaccccggcgagagcccccttctccccacatatcaaacctcccccggttcccacacttgccgttaagggcgtagggtactgcagtctggaatctacgcttgttcagactttgtactagtttctttgtctggccatccgggtaacccatgccggacgcaaaatagactactgaaaatttttttgctttgtggttgggactttagccaagggtataaaagaccaccgtccccgaattacctttcctcttcttttctctctctccttgtcaactcacacccgaaatcgttaagcatttccttctgagtataagaatcattcaaaatggtgagtttcagaggcagcagcaattgccacgggctttgagcacacggccgggtgtggtcccattcccatcgacacaagacgccacgtcatccgaccagcactttttgcagtactaaccgcaggattataacagcgcggatttcaaggagatatggggcaaggccgccgacaccgcgctgctgggaccgtacaactacctcgccaacaaccggggccacaacatcagagaacacttgatcgcagcgttcggagcggttatcaaggtggacaagagcgatctcgagaccatttcgcacatcaccaagattttgcataactcgtcgctgcttgttgatgacgtggaagacaactcgatgctccgacgaggcctgccggcagcccattgtctgtttggagtcccccaaaccatcaactccgccaactacatgtactttgtggctctgcaggaggtgctcaagctcaagtcttatgatgccgtctccattttcaccgaggaaatgatcaacttgcatagaggtcagggtatggatctctactggagagaaacactcacttgcccctcggaagacgagtatctggagatggtggtgcacaagaccggtggactgtttcggctggctctgagacttatgctgtcggtggcatcgaaacaggaggaccatgaaaagatcaactttgatctcacacaccttaccgacacactgggagtcatttaccagattctggatgattacctcaacctgcagtccacggaattgaccgagaacaagggattctgcgaagatatcagcgaaggaaagttttcgtttccgctgattcacagcatacgcaccaacccggataaccacgagattctcaacattctcaaacagcgaacaagcgacgcttcactcaaaaagtacgccgtggactacatgagaacagaaaccaagagtttcgactactgcctcaagaggatacaggccatgtcactcaaggcaagttcgtacattgatgatctagcagcagctggccacgatgtctccaagctacgagccattttgcattattttgtgtccacctctgactgtgaggagagaaagtactttgaggatgcgcagtgactatccgaagatcaagagcgaagcaagttgtaagtccaggacatgtttcccgcccacgcgagtgatttataacacctctcttttttgacacccgctcgccttgaaattcatgtcacataaattatagtcaacgacgtttgaataacttgtcttgtagttcgatgatgatcatatgattacattaatagtaattactgtatttgatatatatactaattacaatagtacatattagaacatacaatagttagtgccgtgaagtggcttaaaataccgcgagtcgattacgtaatattatatataatgtcaaagtggggtcccagagccgaagaaggtgcttttcttgaagatcccagtgtattggacaagtatatctgtctctatgattgtttttccaggtgaaaatgttgaacaaagtgtctactggagtttgtaagcgctggtgcgactggggccacttttaaaacccgccttagcaggctttttcaccgttccaagac

SEQ ID NO: 12 - DNA, 828 bp, synthetic construct
  source 1..828: mol_type = other DNA
atgggcctgatgctgatcgactggtgtgccctggccctggtggtgttcatcggcctgccccacggcgccctggacgccgccatctctttctctatgatctcttctgccaagcgaatcgcccgactggccggcatcctgctgatctacctgctgctggccaccgccttcttcctgatctggtaccagctgcccgccttctctctgctgatcttcctgctgatctctatcatccacttcggcatggccgacttcaacgcctctccctctaagctgaagtggccccacatcatcgcccacggcggcgtggtgaccgtgtggctgcccctgatccagaagaacgaggtgaccaagctgttctctatcctgaccaacggccccacccccatcctgtgggacatcctgctgatcttcttcctgtgttggtctatcggcgtgtgtctgcacacctacgagaccctgcgatctaagcactacaacatcgccttcgagctgatcggcctgatcttcctggcctggtacgccccccccctggtgaccttcgccacctacttctgtttcatccactctcgacgacacttctctttcgtgtggaagcagctgcagcacatgtcttctaagaagatgatgatcggctctgccatcatcctgtcttgtacctcttggctgatcggcggcggcatctacttcttcctgaactctaagatgatcgcctctgaggccgccctgcagaccgtgttcatcggcctggccgccctgaccgtgccccacatgatcctgatcgacttcatcttccgaccccactcttctcgaatcaagatcaagaactag

SEQ ID NO: 13 - DNA, 254 bp, synthetic construct
  source 1..254: mol_type = other DNA
ctcgagtcatgtaattagttatgtcacgcttacattcacgccctccccccacatccgctctaaccgaaaaggaaggagttagacaacctgaagtctaggtccctatttatttttttatagttatgttagtattaagaacgttatttatatttcaaatttttcttttttttctgtacagacgcgtgtacgcatgtaacattatactgaaaaccttgcttgagaaggttttgggacgctcgaaggctttaatttgc

SEQ ID NO: 14 - DNA, 1610 bp, synthetic construct
  source 1..1610: mol_type = other DNA
agagaccgggttggcggcgcatttgtgtcccaaaaaacagccccaattgccccaattgaccccaaattgacccagtagcgggcccaaccccggcgagagcccccttctccccacatatcaaacctcccccggttcccacacttgccgttaagggcgtagggtactgcagtctggaatctacgcttgttcagactttgtactagtttctttgtctggccatccgggtaacccatgccggacgcaaaatagactactgaaaatttttttgctttgtggttgggactttagccaagggtataaaagaccaccgtccccgaattacctttcctcttcttttctctctctccttgtcaactcacacccgaaatcgttaagcatttccttctgagtataagaatcattcaaaatggtgagtttcagaggcagcagcaattgccacgggctttgagcacacggccgggtgtggtcccattcccatcgacacaagacgccacgtcatccgaccagcactttttgcagtactaaccgcagggcctgatgctgatcgactggtgtgccctggccctggtggtgttcatcggcctgccccacggcgccctggacgccgccatctctttctctatgatctcttctgccaagcgaatcgcccgactggccggcatcctgctgatctacctgctgctggccaccgccttcttcctgatctggtaccagctgcccgccttctctctgctgatcttcctgctgatctctatcatccacttcggcatggccgacttcaacgcctctccctctaagctgaagtggccccacatcatcgcccacggcggcgtggtgaccgtgtggctgcccctgatccagaagaacgaggtgaccaagctgttctctatcctgaccaacggccccacccccatcctgtgggacatcctgctgatcttcttcctgtgttggtctatcggcgtgtgtctgcacacctacgagaccctgcgatctaagcactacaacatcgccttcgagctgatcggcctgatcttcctggcctggtacgccccccccctggtgaccttcgccacctacttctgtttcatccactctcgacgacacttctctttcgtgtggaagcagctgcagcacatgtcttctaagaagatgatgatcggctctgccatcatcctgtcttgtacctcttggctgatcggcggcggcatctacttcttcctgaactctaagatgatcgcctctgaggccgccctgcagaccgtgttcatcggcctggccgccctgaccgtgccccacatgatcctgatcgacttcatcttccgaccccactcttctcgaatcaagatcaagaactagctcgagtcatgtaattagttatgtcacgcttacattcacgccctccccccacatccgctctaaccgaaaaggaaggagttagacaacctgaagtctaggtccctatttatttttttatagttatgttagtattaagaacgttatttatatttcaaatttttcttttttttctgtacagacgcgtgtacgcatgtaacattatactgaaaaccttgcttgagaaggttttgggacgctcgaaggctttaatttgc

SEQ ID NO: 15 - DNA, 24 bp, synthetic construct
  source 1..24: mol_type = other DNA
catcatttcaaaagagggaacagc

SEQ ID NO: 16 - DNA, 41 bp, synthetic construct
  source 1..41: mol_type = other DNA
cgccgccaacccggtctctgtgtttggcggtgtgagttgtc

SEQ ID NO: 17 - DNA, 41 bp, synthetic construct
  source 1..41: mol_type = other DNA
gacaactcacaccgccaaacacagagaccgggttggcggcg

SEQ ID NO: 18 - DNA, 45 bp, synthetic construct
  source 1..45: mol_type = other DNA
agctgcatctggtgggcagcctgcggttagtactgcaaaaagtgc

SEQ ID NO: 19 - DNA, 45 bp, synthetic construct
  source 1..45: mol_type = other DNA
gcactttttgcagtactaaccgcaggctgcccaccagatgcagct

SEQ ID NO: 20 - DNA, 40 bp, synthetic construct
  source 1..40: mol_type = other DNA
cgctcttgatcttcggatagtcagttctgtcggtatccga

SEQ ID NO: 21 - DNA, 40 bp, synthetic construct
  source 1..40: mol_type = other DNA
tcggataccgacagaactgactatccgaagatcaagagcg

SEQ ID NO: 22 - DNA, 45 bp, synthetic construct
  source 1..45: mol_type = other DNA
gacgagtcagacaggaggcagtcttggaacggtgaaaaagcctgc

SEQ ID NO: 23 - DNA, 45 bp, synthetic construct
  source 1..45: mol_type = other DNA
gcaggctttttcaccgttccaagactgcctcctgtctgactcgtc

SEQ ID NO: 24 - DNA, 41 bp, synthetic construct
  source 1..41: mol_type = other DNA
cgctcttgatcttcggatagtggtggtattgtgactgggga

SEQ ID NO: 25 - DNA, 41 bp, synthetic construct
  source 1..41: mol_type = other DNA
tccccagtcacaataccaccactatccgaagatcaagagcg

SEQ ID NO: 26 - DNA, 48 bp, synthetic construct
  source 1..48: mol_type = other DNA
catatggagtgttatttgaaggggtcttggaacggtgaaaaagcctgc

SEQ ID NO: 27 - DNA, 48 bp, synthetic construct
  source 1..48: mol_type = other DNA
gcaggctttttcaccgttccaagaccccttcaaataacactccatatg

SEQ ID NO: 28 - DNA, 21 bp, synthetic construct
  source 1..21: mol_type = other DNA
ccgatacagtgtccaagtacg

SEQ ID NO: 29 - DNA, 22 bp, synthetic construct
  source 1..22: mol_type = other DNA
gagtgtctgaagacaaggcttc

SEQ ID NO: 30 - DNA, 20 bp, synthetic construct
  source 1..20: mol_type = other DNA
gacgacaatgctgagctccg

SEQ ID NO: 31 - DNA, 47 bp, synthetic construct
  source 1..47: mol_type = other DNA
ctgtgaggatgttcgcgtaatcctgcggttagtactgcaaaaagtgc

SEQ ID NO: 32 - DNA, 47 bp, synthetic construct
  source 1..47: mol_type = other DNA
gcactttttgcagtactaaccgcaggattacgcgaacatcctcacag

SEQ ID NO: 33 - DNA, 44 bp, synthetic construct
  source 1..44: mol_type = other DNA
cttcgctcttgatcttcggatagtcacagagggatatcggctag

SEQ ID NO: 34 - DNA, 44 bp, synthetic construct
  source 1..44: mol_type = other DNA
ctagccgatatccctctgtgactatccgaagatcaagagcgaag

SEQ ID NO: 35 - DNA, 46 bp, synthetic construct
  source 1..46: mol_type = other DNA
cagctcatctatcttggcctcctgcggttagtactgcaaaaagtgc

SEQ ID NO: 36 - DNA, 46 bp, synthetic construct
  source 1..46: mol_type = other DNA
gcactttttgcagtactaaccgcaggaggccaagatagatgagctg

SEQ ID NO: 37 - DNA, 57 bp, synthetic construct
  source 1..57: mol_type = other DNA
cttcgctcttgatcttcggatagtcacaattcggataagtggtctattatatataac

SEQ ID NO: 38 - DNA, 57 bp, synthetic construct
  source 1..57: mol_type = other DNA
gttatatataatagaccacttatccgaattgtgactatccgaagatcaagagcgaag

SEQ ID NO: 39 - DNA, 49 bp, synthetic construct
  source 1..49: mol_type = other DNA
cttgaaatccgcgctgttataatcctgcggttagtactgcaaaaagtgc

SEQ ID NO: 40 - DNA, 49 bp, synthetic construct
  source 1..49: mol_type = other DNA
gcactttttgcagtactaaccgcaggattataacagcgcggatttcaag

SEQ ID NO: 41 - DNA, 45 bp, synthetic construct
  source 1..45: mol_type = other DNA
cttcgctcttgatcttcggatagtcactgcgcatcctcaaagtac

SEQ ID NO: 42 - DNA, 45 bp, synthetic construct
  source 1..45: mol_type = other DNA
gtactttgaggatgcgcagtgactatccgaagatcaagagcgaag

SEQ ID NO: 43 - DNA, 25 bp, synthetic construct
  source 1..25: mol_type = other DNA
ggcgtttcaggtggttgcgtgagtg

SEQ ID NO: 44 - DNA, 53 bp, synthetic construct
  source 1..53: mol_type = other DNA
gacacaaatgcgccgccaacccggtctctgcggcggttcgtggttcgtgtttc

SEQ ID NO: 45 - DNA, 53 bp, synthetic construct
  source 1..53: mol_type = other DNA
gaaacacgaaccacgaaccgccgcagagaccgggttggcggcgcatttgtgtc

SEQ ID NO: 46 - DNA, 40 bp, synthetic construct
  source 1..40: mol_type = other DNA
cagtcgatcagcatcaggccctgcggttagtactgcaaaa

SEQ ID NO: 47 - DNA, 40 bp, synthetic construct
  source 1..40: mol_type = other DNA
ttttgcagtactaaccgcagggcctgatgctgatcgactg

SEQ ID NO: 48 - DNA, 40 bp, synthetic construct
  source 1..40: mol_type = other DNA
aactaattacatgactcgagctagttcttgatcttgattc

SEQ ID NO: 49 - DNA, 40 bp, synthetic construct
  source 1..40: mol_type = other DNA
gaatcaagatcaagaactagctcgagtcatgtaattagtt

SEQ ID NO: 50 - DNA, 45 bp, synthetic construct
  source 1..45: mol_type = other DNA
gacgagtcagacaggaggcagcaaattaaagccttcgagcgtccc

SEQ ID NO: 51 - DNA, 45 bp, synthetic construct
  source 1..45: mol_type = other DNA
gggacgctcgaaggctttaatttgctgcctcctgtctgactcgtc

SEQ ID NO: 52 - DNA, 40 bp, synthetic construct
  source 1..40: mol_type = other DNA
aactaattacatgactcgagtggtggtattgtgactgggg

SEQ ID NO: 53 - DNA, 40 bp, synthetic construct
  source 1..40: mol_type = other DNA
ccccagtcacaataccaccactcgagtcatgtaattagtt

SEQ ID NO: 54 - DNA, 48 bp, synthetic construct
  source 1..48: mol_type = other DNA
gcagcagtcatacatgttctgaggcaaattaaagccttcgagcgtccc

SEQ ID NO: 55 - DNA, 48 bp, synthetic construct
  source 1..48: mol_type = other DNA
gggacgctcgaaggctttaatttgcctcagaacatgtatgactgctgc

SEQ ID NO: 56 - DNA, 25 bp, synthetic construct
  source 1..25: mol_type = other DNA
ctactttgtgcagattgaggccaag

SEQ ID NO: 57 - DNA, 20 bp, synthetic construct
  source 1..20: mol_type = other DNA
gtcgtctgtcttctcttcag

SEQ ID NO: 58 - DNA, 20 bp, synthetic construct
  source 1..20: mol_type = other DNA
ccaccaagatgggcaagaag

SEQ ID NO: 59 - DNA, 2022 bp, Xanthophyllomyces dendrorhous
  source 1..2022: mol_type = genomic DNA
atgacggctctcgcatattaccagatccatctgatctatactctcccaattcttggtcttctcggcctgctcacttccccgattttgacaaaatttgacatctacaaaatatcgatcctcgtatttattgcgtttagtgcaaccacaccatgggactcatggatcatcagaaatggcgcatggacatatccatcagcggagagtggccaaggcgtgtttggaacgtttctagatgttccatatgaagagtacgctttctttgtcattcaaaccgtaatcaccggcttggtctacgtcttggcaactaggcaccttctcccatctctcgcgcttcccaagactagatcgtccgccctttctctcgcgctcaaggcgctcatccctctgcccattatctacctatttaccgctcaccccagcccatcgcccgacccgctcgtgacagatcactacttctacatgcgggcactctccttactcatcaccccacctaccatgctcttggcagcattatcaggcgaatatgctttcgattggaaaagtggccgagcaaagtcaactattgcagcaatcatgatcccgacggtgtatctgatttgggtagattatgttgctgtcggtcaagactcttggtcgatcaacgatgagaagattgtagggtggaggcttggaggtgtactacccattgaggaagctatgttcttcttactgacgaatctaatgattgttctgggtctgtctgcctgcgatcatactcaggccctatacctgctacacggtcgaactatttatggcaacaaaaagatgccatcttcatttcccctcattacaccgcctgtgctctccctgttttttagcagccgaccatactcttctcagccaaaacgtgacttggaactggcagtcaagttgttggaggaaaagagccggagcttttttgttgcctcggctggatttcctagcgaagttagggagaggctggttggactatacgcattctgccgggtgactgatgatcttatcgactctcctgaagtatcttccaacccgcatgccacaattgacatggtctccgattttcttaccctactatttgggcccccgctacacccttcgcaacctgacaagatcctttcttcgcctttacttcctccttcgcacccttcccgacccacgggaatgtatcccctcccgcctcctccttcgctctcgcctgccgagctcgttcaattccttaccgaaagggttcccgttcaataccatttcgccttcaggttgctcgctaagttgcaagggctgatccctcgatacccactcgacgaactccttagaggatacaccactgatcttatctttcccttatcgacagaggcagtccaggctcggaagacgcctatcgagaccacagctgacttgctggactatggtctatgtgtagcaggctcagtcgccgagctattggtctatgtctcttgggcaagtgcaccaagtcaggtccctgccaccatagaagaaagagaagctgtgttagtggcaagccgagagatgggaactgcccttcagttggtgaacattgctagggacattaaaggggacgcaacagaagggagattttacctaccactctcattctttggtcttcgggatgaatcaaagcttgcgatcccgactgattggacggaacctcggcctcaagatttcgacaaactcctcagtctatctccttcgtccacattaccatcttcaaacgcctcagaaagcttccggttcgaatggaagacgtactcgcttccattagtcgcctacgcagaggatcttgccaaacattcttataagggaattgaccgacttcctaccgaggttcaagcgggaatgcgagcggcttgcgcgagctacctactgatcggccgagagatcaaagtcgtttggaaaggagacgtcggagagagaaggacagttgccggatggaggagagtacggaaagtcttgagtgtggtcatgagcggatgggaagggcagtaa

SEQ ID NO: 60 - DNA, 1749 bp, Xanthophyllomyces dendrorhous
  source 1..1749: mol_type = genomic DNA
atgggaaaagaacaagatcaggataaacccacagctatcatcgtgggatgtggtatcggtggaatcgccactgccgctcgtcttgctaaagaaggtttccaggtcacggtgttcgagaagaacgactactccggaggtcgatgctctttaatcgagcgagatggttatcgattcgatcaggggcccagtttgctgctcttgccagatctcttcaagcagacattcgaagatttgggagagaagatggaagattgggtcgatctcatcaagtgtgaacccaactatgtttgccacttccacgatgaagagactttcactctttcaaccgacatggcgttgctcaagcgggaagtcgagcgttttgaaggcaaagatggatttgatcggttcttgtcgtttatccaagaagcccacagacattacgagcttgctgtcgttcacgtcctgcagaagaacttccctggcttcgcagcattcttacggctacagttcattggccaaatcctggctcttcaccccttcgagtctatctggacaagagtttgtcgatatttcaagaccgacagattacgaagagtcttctcgtttgcagtgatgtacatgggtcaaagcccatacagtgcgcccggaacatattccttgctccaatacaccgaattgaccgagggcatctggtatccgagaggaggcttttggcaggttcctaatactcttcttcagatcgtcaagcgcaacaatccctcagccaagttcaatttcaacgctccagtttcccaggttcttctctctcctgccaaggaccgagcgactggtgttcgacttgaatccggcgaggaacatcacgccgatgttgtgattgtcaatgctgacctcgtttacgcctccgagcacttgattcctgacgatgccagaaacaagattggccaactgggtgaagtcaagagaagttggtgggctgacttagttggtggaaagaagctcaagggaagttgcagtagtttgagcttctactggagcatggaccgaatcgtggacggtctgggcggacacaatatcttcttggccgaggacttcaagggatcattcgacacaatcttcgaggagttgggtctcccagccgatccttccttttacgtgaacgttccctcgcgaatcgatccttctgccgctcccgaaggcaaagatgctatcgtcattcttgtgccgtgtggccatatcgacgcttcgaaccctcaagattacaacaagcttgttgctcgggcaaggaagtttgtgatccacacgctttccgccaagcttggacttcccgactttgaaaaaatgattgtggcagagaaggttcacgatgctccctcttgggagaaagaattcaacctcaaggacggaagcatcttgggactggctcacaactttatgcaagttcttggtttcaggccgagcaccagacatcccaagtatgacaagttgttctttgtcggggcttcgactcatcccggaactggggttcccatcgtcttggctggagccaagttaactgccaaccaagttctcgaatcctttgaccgatccccagctccagatcccaatatgtcactctccgtaccatatggaaaacctctcaaatcaaatggaacgggtatcgattctcaggtccagctgaagttcatggatttggagagatgggtataccttttggtgttgttgattggggccgtgatcgctcgatccgttggtgttcttgctttctga

SEQ ID NO: 61 - DNA, 2804 bp, synthetic construct
  source 1..2804: mol_type = other DNA
agagaccgggttggcggcgcatttgtgtcccaaaaaacagccccaattgccccaattgaccccaaattgacccagtagcgggcccaaccccggcgagagcccccttctccccacatatcaaacctcccccggttcccacacttgccgttaagggcgtagggtactgcagtctggaatctacgcttgttcagactttgtactagtttctttgtctggccatccgggtaacccatgccggacgcaaaatagactactgaaaatttttttgctttgtggttgggactttagccaagggtataaaagaccaccgtccccgaattacctttcctcttcttttctctctctccttgtcaactcacacccgaaatcgttaagcatttccttctgagtataagaatcattcaaaatggtgagtttcagaggcagcagcaattgccacgggctttgagcacacggccgggtgtggtcccattcccatcgacacaagacgccacgtcatccgaccagcactttttgcagtactaaccgcagacggctctcgcatattaccagatccatctgatctatactctcccaattcttggtcttctcggtctgctcacttccccgattttgacaaaatttgacatctacaaaatatcgatcctcgtatttattgcgtttagtgcaaccacaccatgggactcatggatcatcagaaatggcgcatggacatatccatcagcggagagtggccaaggcgtgtttggaacgtttctagatgttccatatgaagagtacgctttctttgtcattcaaaccgtaatcaccggcttggtctacgtcttggcaactaggcaccttctcccatctctcgcgcttcccaagactagatcgtccgccctttctctcgcgctcaaggcgctcatccctctgcccattatctacctatttaccgctcaccccagcccatcgcccgacccgctcgtgacagatcactacttctacatgcgggcactctccttactcatcaccccacctaccatgctcttggcagcattatcaggcgaatatgctttcgattggaaaagtggccgagcaaagtcaactattgcagcaatcatgatcccgacggtgtatctgatttgggtagattatgttgctgtcggtcaagactcttggtcgatcaacgatgagaagattgtagggtggaggcttggaggtgtactacccattgaggaagctatgttcttcttactgacgaatctaatgattgttctgggtctgtctgcctgcgatcatactcaggccctatacctgctacacggtcgaactatttatggcaacaaaaagatgccatcttcatttcccctcattacaccgcctgtgctctccctgttttttagcagccgaccatactcttctcagccaaaacgtgacttggaactggcagtcaagttgttggaggaaaagagccggagcttttttgttgcctcggctggatttcctagcgaagttagggagaggctggttggactatacgcattctgccgggtgactgatgatcttatcgactctcctgaagtatcttccaacccgcatgccacaattgacatggtctccgattttcttaccctactatttgggcccccgctacacccttcgcaacctgacaagatcctttcttcgcctttacttcctccttcgcacccttcccgacccacgggaatgtatcccctcccgcctcctccttcgctctcgcctgccgagctcgttcaattccttaccgaaagggttcccgttcaataccatttcgccttcaggttgctcgctaagttgcaagggctgatccctcgatacccactcgacgaactccttagaggatacaccactgatcttatctttcctttatcgacagaggcagtccaggctcggaagacgcctatcgagaccacagctgacttgctggactatggtctatgtgtagcaggctcagtcgccgagctattggtctatgtctcttgggcaagtgcaccaagtcaggtccctgccaccatagaagaaagagaagctgtgttagtggcaagccgagagatgggaactgcccttcagttggtgaacattgctagggacattaaaggggacgcaacagaagggagattttacctaccactctcattctttggtcttcgggatgaatcaaagcttgcgatcccgactgattggacggaacctcggcctcaagatttcgacaaactcctcagtctatctccttcgtccacattaccatcttcaaacgcctcagaaagcttccggttcgaatggaagacgtactcgcttccattagtcgcctacgcagaggatcttgccaaacattcttataagggaattgaccgacttcctaccgaggttcaagcgggaatgcgagcggcttgcgcgagctacctactgatcggccgagagatcaaagtcgtttggaaaggagacgtcggagagagaaggacagttgccggatggaggagagtacggaaagtcttgagtgtggtcatgagcggatgggaagggcagtaactcgagtcatgtaattagttatgtcacgcttacattcacgccctccccccacatccgctctaaccgaaaaggaaggagttagacaacctgaagtctaggtccctatttatttttttatagttatgttagtattaagaacgttatttatatttcaaatttttcttttttttctgtacagacgcgtgtacgcatgtaacattatactgaaaaccttgcttgagaaggttttgggacgctcgaaggctttaatttgc

SEQ ID NO: 62 - DNA, 2531 bp, synthetic construct
  source 1..2531: mol_type = other DNA
agagaccgggttggcggcgcatttgtgtcccaaaaaacagccccaattgccccaattgaccccaaattgacccagtagcgggcccaaccccggcgagagcccccttctccccacatatcaaacctcccccggttcccacacttgccgttaagggcgtagggtactgcagtctggaatctacgcttgttcagactttgtactagtttctttgtctggccatccgggtaacccatgccggacgcaaaatagactactgaaaatttttttgctttgtggttgggactttagccaagggtataaaagaccaccgtccccgaattacctttcctcttcttttctctctctccttgtcaactcacacccgaaatcgttaagcatttccttctgagtataagaatcattcaaaatggtgagtttcagaggcagcagcaattgccacgggctttgagcacacggccgggtgtggtcccattcccatcgacacaagacgccacgtcatccgaccagcactttttgcagtactaaccgcagggaaaagaacaagatcaggataaacccacagctatcatcgtgggatgtggtatcggtggaatcgccactgccgctcgtcttgctaaagaaggtttccaggtcacggtgttcgagaagaacgactactccggaggtcgatgctctttaatcgagcgagatggttatcgattcgatcaggggcccagtttgctgctcttgccagatctcttcaagcagacattcgaagatttgggagagaagatggaagattgggtcgatctcatcaagtgtgaacccaactatgtttgccacttccacgatgaagagactttcactctttcaaccgacatggcgttgctcaagcgggaagtcgagcgttttgaaggcaaagatggatttgatcggttcttgtcgtttatccaagaagcccacagacattacgagcttgctgtcgttcacgtcctgcagaagaacttccctggcttcgcagcattcttacggctacagttcattggccaaatcctggctcttcaccccttcgagtctatctggacaagagtttgtcgatatttcaagaccgacagattacgaagagtcttctcgtttgcagtgatgtacatgggtcaaagcccatacagtgcgcccggaacatattccttgctccaatacaccgaattgaccgagggcatctggtatccgagaggaggcttttggcaggttcctaatactcttcttcagatcgtcaagcgcaacaatccctcagccaagttcaatttcaacgctccagtttcccaggttcttctctctcctgccaaggaccgagcgactggtgttcgacttgaatccggcgaggaacatcacgccgatgttgtgattgtcaatgctgacctcgtttacgcctccgagcacttgattcctgacgatgccagaaacaagattggccaactgggtgaagtcaagagaagttggtgggctgacttagttggtggaaagaagctcaagggaagttgcagtagtttgagcttctactggagcatggaccgaatcgtggacggtctgggcggacacaatatcttcttggccgaggacttcaagggatcattcgacacaatcttcgaggagttgggtctcccagccgatccttccttttacgtgaacgttccctcgcgaatcgatccttctgccgctcccgaaggcaaagatgctatcgtcattcttgtgccgtgtggccatatcgacgcttcgaaccctcaagattacaacaagcttgttgctcgggcaaggaagtttgtgatccacacgctttccgccaagcttggacttcccgactttgaaaaaatgattgtggcagagaaggttcacgatgctccctcttgggagaaagaattcaacctcaaggacggaagcatcttgggactggctcacaactttatgcaagttcttggtttcaggccgagcaccagacatcccaagtatgacaagttgttctttgtcggggcttcgactcatcccggaactggggttcccatcgtcttggctggagccaagttaactgccaaccaagttctcgaatcctttgaccgatccccagctccagatcccaatatgtcactctccgtaccatatggaaaacctctcaaatcaaatggaacgggtatcgattctcaggtccagctgaagttcatggatttggagagatgggtataccttttggtattgttgattggggccgtgatcgctcgatccgttggtgttcttgctttctgactcgagtcatgtaattagttatgtcacgcttacattcacgccctccccccacatccgctctaaccgaaaaggaaggagttagacaacctgaagtctaggtccctatttatttttttatagttatgttagtattaagaacgttatttatatttcaaatttttcttttttttctgtacagacgcgtgtacgcatgtaacattatactgaaaaccttgcttgagaaggttttgggacgctcgaaggctttaatttgc

SEQ ID NO: 63 - DNA, 1533 bp, Yarrowia lipolytica; identical to SEQ ID NO: 5
  source 1..1533: mol_type = genomic DNA

SEQ ID NO: 64 - DNA, 30 bp, synthetic construct
  source 1..30: mol_type = other DNA
gtgcgcttctctcgtctcggtaaccctgtc

SEQ ID NO: 65 - DNA, 44 bp, synthetic construct
  source 1..44: mol_type = other DNA
atgcgccgccaacccggtctctggggtgtggtggatggggtgtg

SEQ ID NO: 66 - DNA, 44 bp, synthetic construct
  source 1..44: mol_type = other DNA
cacaccccatccaccacaccccagagaccgggttggcggcgcat

SEQ ID NO: 67 - DNA, 39 bp, synthetic construct
  source 1..39: mol_type = other DNA
cgccgccaacccggtctcttgaagacgaaagggcctccg

SEQ ID NO: 68 - DNA, 39 bp, synthetic construct
  source 1..39: mol_type = other DNA
cggaggccctttcgtcttcaagagaccgggttggcggcg

SEQ ID NO: 69 - DNA, 40 bp, synthetic construct
  source 1..40: mol_type = other DNA
gacgagtcagacaggaggcatcagacagatactcgtcgcg

SEQ ID NO: 70 - DNA, 40 bp, synthetic construct
  source 1..40: mol_type = other DNA
cgcgacgagtatctgtctgatgcctcctgtctgactcgtc

SEQ ID NO: 71 - DNA, 44 bp, synthetic construct
  source 1..44: mol_type = other DNA
atgacgagtcagacaggaggcatggtggtattgtgactggggat

SEQ ID NO: 72 - DNA, 44 bp, synthetic construct
  source 1..44: mol_type = other DNA
atccccagtcacaataccaccatgcctcctgtctgactcgtcat

SEQ ID NO: 73 - DNA, 44 bp, synthetic construct
  source 1..44: mol_type = other DNA
cggcgtccttctcgtagtccgcttttggtggtgaagaggagact

SEQ ID NO: 74 - DNA, 44 bp, synthetic construct
  source 1..44: mol_type = other DNA
agtctcctcttcaccaccaaaagcggactacgagaaggacgccg

SEQ ID NO: 75 - DNA, 30 bp, synthetic construct
  source 1..30: mol_type = other DNA
ccactcgtcaccaacagtgccgtgtgttgc

SEQ ID NO: 76 - DNA, 24 bp, synthetic construct
  source 1..24: mol_type = other DNA
tcgtacgtctataccaacagatgg

SEQ ID NO: 77 - DNA, 24 bp, synthetic construct
  source 1..24: mol_type = other DNA
cgcatacacacacactgccggggg

SEQ ID NO: 78 - DNA, 550 bp, Yarrowia lipolytica
  source 1..550: mol_type = genomic DNA
tccacacgtcgttcttttttccttagccttttttgcagtgcgcgtgtcccaaaccccagctctacacaccagcacaaacaaagttaagctcagggttgtcgttgaggtcgcttactgtagtcagtgctcgtatggttcgttcaattttcgccaaaaatcgttttgcctttgtatcttgggaataacatcaactgtggttcttcaacaggcctaaggaacgaaacaagccggaccaagatcaggttcaaggtgagtactgagaaggaatagaaggcctaaaggcgcaaaccgacaggtggcaacagctccacaccgaccacgaaggccacgaaatcaaggggtcctaaagttagtctttgtggcctcgacggtcagcgaaaacgcgagaccacaacgcgatcagaaccaggacctaaacaacacaggacggggtcacaataggcttgaacagcaagtacaagctgtgatctctctatatttgattctcaaaccacccctgactacttcagcgcctctgtgacacagcccccctatcatccgactaacacag

SEQ ID NO: 79 - DNA, 31 bp, synthetic construct
  source 1..31: mol_type = other DNA
gacaatgcctcgaggaggtttaaaagtaact

SEQ ID NO: 80 - DNA, 41 bp, synthetic construct
  source 1..41: mol_type = other DNA
gcgccgccaacccggtctctctgtgttagtcggatgatagg

SEQ ID NO: 81 - DNA, 41 bp, synthetic construct
  source 1..41: mol_type = other DNA
cctatcatccgactaacacagagagaccgggttggcggcgc

SEQ ID NO: 82 - DNA, 42 bp, synthetic construct
  source 1..42: mol_type = other DNA
gacgagtcagacaggaggcactgcggttagtactgcaaaaag

SEQ ID NO: 83 - DNA, 42 bp, synthetic construct
  source 1..42: mol_type = other DNA
ctttttgcagtactaaccgcagtgcctcctgtctgactcgtc

SEQ ID NO: 84 - DNA, 44 bp, synthetic construct
  source 1..44: mol_type = other DNA
atgcgccgccaacccggtctcttggtggtattgtgactggggat

SEQ ID NO: 85 - DNA, 44 bp, synthetic construct
  source 1..44: mol_type = other DNA
atccccagtcacaataccaccaagagaccgggttggcggcgcat

SEQ ID NO: 86 - DNA, 41 bp, synthetic construct
  source 1..41: mol_type = other DNA
ctttccaatagctgcttgtagctgcggttagtactgcaaaa

SEQ ID NO: 87 - DNA, 41 bp, synthetic construct
  source 1..41: mol_type = other DNA
ttttgcagtactaaccgcagctacaagcagctattggaaag

SEQ ID NO: 88 - DNA, 30 bp, synthetic construct
  source 1..30: mol_type = other DNA
gcttaatgtgattgatctcaaacttgatag

SEQ ID NO: 89 - DNA, 24 bp, synthetic construct
  source 1..24: mol_type = other DNA
gctgtctctgcgagagcacgtcga

SEQ ID NO: 90 - DNA, 24 bp, synthetic construct
  source 1..24: mol_type = other DNA
ggttcgcacaacttctcgggtggc

SEQ ID NO: 91 - protein, 357 aa, Dunaliella salina
MAAHQMQLLNSQRLCSTSTRSIRPAVSNRPQVPRRPANVRRGRYQACRTMAIATADEAKQSTSSFDFQGYMMERAVMVNDALDKALPQRHPEVLLDAMRYSLLAGGKRVRPALTLAACELVGGDIACAMPTACAMEVVHTMSLIHDDLPSMDNDDFRRGRPTNHKVYGEDIAILAGDALLSFAFEHVARATTGTSPERVLRVILELGKAVGADGLTGGQVVDIKSENEEVGLEVLQYIHEHKTAALLEASVVCGALVGGADDVTVEKLRKYARNIGLAFQVVDDILDCTQTTEMLGKTAGKDIDVNKTTYPKLLGLEKSKQAAEDLIAEAIQQLDGFPPEKRTPLVALAKYIGYRQN